European Patent Application EP 4 335 864 A1, published March 13, 2024. Title: Interferon inhibitor and its use in the treatment of autoinflammatory diseases. Applicant: CONSEJO SUPERIOR DE INVESTIGACIONES CIENTIFICAS (CISC). The sequence listing filed with the application follows.

SEQUENCE LISTING (37 sequences)

SEQ ID NO: 1 - protein, 100 aa, Vaccinia virus
FKLILDPKINVTIGEPANITCTAVSTSLLIDDVLIEWENPSGWLIGFDFDVYSVLTSRGGITEATLYFENVTEEYIGNTYKCRGHNYYFEKTLTTTVVLE

SEQ ID NO: 2 - protein, 254 aa, synthetic construct
MTMKMMVHIYFVSLLLLLFHSYAIDIENEITEFFNKMRDTLPAKDSKWLNPAPPSCIPKTYELGTHDKYGIDLYCGILYAKHYNNITWYKDNKEINIDDIKYSQTGKELIIHNPELEDSGRYDCYVHYDDVRIKNDIVVSRCKILTVIPSQDHRFKLILDPKINVTIGEPANITCTAVSTSLLIDDVLIEWENPSGWLIGFDFDVYSVLTSRGGITEATLYFENVTEEYIGNTYKCRGHNYYFEKTLTTTVVLE

SEQ ID NO: 3 - protein, 203 aa, synthetic construct
MPPSCIPKTYELGTHDKYGIDLYCGILYAKHYNNITWYKDNKEINIDDIKYSQTGKELIIHNPELEDSGRYDCYVHYDDVRIKNDIVVSRCKILTVIPSQDHRFKLILDPKINVTIGEPANITCTAVSTSLLIDDVLIEWENPSGWLIGFDFDVYSVLTSRGGITEATLYFENVTEEYIGNTYKCRGHNYYFEKTLTTTVVLE

SEQ ID NO: 4 - protein, 59 aa, Vaccinia virus
KWERLEKNRRRQVSNKRVKHGDLWIANYTSKFSNRRYLCTVTTKNGDCVQGIVRSHIRK

SEQ ID NO: 5 - protein, 128 aa, Vaccinia virus
IDIENEITEFFNKMRDTLPAKDSKWLNPACMFGGTMNDIAALGEPFSAKCPPIEDSLLSHRYKDYVVKWERLEKNRRRQVSNKRVKHGDLWIANYTSKFSNRRYLCTVTTKNGDCVQGIVRSHIRKVD

SEQ ID NO: 6 - protein, 65 aa, Molluscum contagiosum virus
PPGAPTSPGAPTLPGAPKVVGTPPPKGNKKNKKKGKGKKRRGNKTKHKNDKKRGGIPKNRHVRVD

SEQ ID NO: 7 - DNA, 177 bp, Vaccinia virus
  source 1..177: mol_type = genomic DNA
aaatgggaaaggctagaaaaaaatagacggcgacaggtttctaataaacgtgttaaacatggtgatttatggatagccaactatacatctaaattcagtaaccgtaggtatttgtgcaccgtaactacaaagaatggtgactgtgttcagggtatagttagatctcatattagaaaa

SEQ ID NO: 8 - DNA, 384 bp, Vaccinia virus
  source 1..384: mol_type = genomic DNA
atagacatcgaaaatgaaatcacagaattcttcaataaaatgagagatactctaccagctaaagactctaaatggttgaatccagcatgtatgttcggaggcacaatgaatgatatagccgctctaggagagccattcagcgcaaagtgtcctcctattgaagacagtcttttatcgcacagatataaagactatgtggttaaatgggaaaggctagaaaaaaatagacggcgacaggtttctaataaacgtgttaaacatggtgatttatggatagccaactatacatctaaattcagtaaccgtaggtatttgtgcaccgtaactacaaagaatggtgactgtgttcagggtatagttagatctcatattagaaaagtcgac

SEQ ID NO: 9 - DNA, 195 bp, Molluscum contagiosum virus
  source 1..195: mol_type = genomic DNA
ccgccgggcgcgccgacgtcaccgggcgcgccaacgctgccgggcgcgccaaaggttgtaggaactccacctccaaaagggaacaagaagaacaagaagaaaggcaaaggaaagaaacgccgcggaaacaagacaaaacacaagaatgataagaaaagggggggcatacccaagaatcgacatgtcagggtcgac

SEQ ID NO: 10 - protein, 15 aa, synthetic construct
  source 1..15: note = Linker
GGGGSGGGGSGGGGS

SEQ ID NO: 11 - protein, 178 aa, synthetic construct
KWERLEKNRRRQVSNKRVKHGDLWIANYTSKFSNRRYLCTVTTKNGDCVQGIVRSHIRKGGGGSGGGGSGGGGSVDHRFKLILDPKINVTIGEPANITCTAVSTSLLIDDVLIEWENPSGWLIGFDFDVYSVLTSRGGITEATLYFENVTEEYIGNTYKCRGHNYYFEKTLTTTVVLE

SEQ ID NO: 12 - DNA, 534 bp, synthetic construct
  source 1..534: mol_type = other DNA
aaatgggaaaggctagaaaaaaatagacggcgacaggtttctaataaacgtgttaaacatggtgatttatggatagccaactatacatctaaattcagtaaccgtaggtatttgtgcaccgtaactacaaagaatggtgactgtgttcagggtatagttagatctcatattagaaaaggtggcggaggttctggtggcggcggtagcggtggcggtggttccgtcgaccacaggtttaaactaatactagatccaaaaatcaacgtaacgataggagaacctgccaatataacatgcactgctgtgtcaacgtcattattgattgacgatgtactgattgaatgggaaaatccatccggatggcttataggattcgattttgatgtatactctgttttaactagtagaggcggtattaccgaggcgaccttgtactttgaaaatgttactgaagaatatataggtaatacatataaatgtcgtggacacaactattattttgaaaaaacccttacaactacagtagtattggag

SEQ ID NO: 13 - protein, 245 aa, synthetic construct
IDIENEITEFFNKMRDTLPAKDSKWLNPACMFGGTMNDIAALGEPFSAKCPPIEDSLLSHRYKDYVVKWERLEKNRRRQVSNKRVKHGDLWIANYTSKFSNRRYLCTVTTKNGDCVQGIVRSHIRKVDGGGGSGGGGSGGGGSHRFKLILDPKINVTIGEPANITCTAVSTSLLIDDVLIEWENPSGWLIGFDFDVYSVLTSRGGITEATLYFENVTEEYIGNTYKCRGHNYYFEKTLTTTVVLE

SEQ ID NO: 14 - DNA, 735 bp, synthetic construct
  source 1..735: mol_type = other DNA
atagacatcgaaaatgaaatcacagaattcttcaataaaatgagagatactctaccagctaaagactctaaatggttgaatccagcatgtatgttcggaggcacaatgaatgatatagccgctctaggagagccattcagcgcaaagtgtcctcctattgaagacagtcttttatcgcacagatataaagactatgtggttaaatgggaaaggctagaaaaaaatagacggcgacaggtttctaataaacgtgttaaacatggtgatttatggatagccaactatacatctaaattcagtaaccgtaggtatttgtgcaccgtaactacaaagaatggtgactgtgttcagggtatagttagatctcatattagaaaagtcgacggtggcggaggttctggtggcggcggtagcggtggcggtggttcccacaggtttaaactaatactagatccaaaaatcaacgtaacgataggagaacctgccaatataacatgcactgctgtgtcaacgtcattattgattgacgatgtactgattgaatgggaaaatccatccggatggcttataggattcgattttgatgtatactctgttttaactagtagaggcggtattaccgaggcgaccttgtactttgaaaatgttactgaagaatatataggtaatacatataaatgtcgtggacacaactattattttgaaaaaacccttacaactacagtagtattggag

SEQ ID NO: 15 - protein, 182 aa, synthetic construct
PPGAPTSPGAPTLPGAPKVVGTPPPKGNKKNKKKGKGKKRRGNKTKHKNDKKRGGIPKNRHVRVDGGGGSGGGGSGGGGSHRFKLILDPKINVTIGEPANITCTAVSTSLLIDDVLIEWENPSGWLIGFDFDVYSVLTSRGGITEATLYFENVTEEYIGNTYKCRGHNYYFEKTLTTTVVLE

SEQ ID NO: 16 - DNA, 546 bp, synthetic construct
  source 1..546: mol_type = other DNA
ccgccgggcgcgccgacgtcaccgggcgcgccaacgctgccgggcgcgccaaaggttgtaggaactccacctccaaaagggaacaagaagaacaagaagaaaggcaaaggaaagaaacgccgcggaaacaagacaaaacacaagaatgataagaaaagggggggcatacccaagaatcgacatgtcagggtcgacggtggcggaggttctggtggcggcggtagcggtggcggtggttcccacaggtttaaactaatactagatccaaaaatcaacgtaacgataggagaacctgccaatataacatgcactgctgtgtcaacgtcattattgattgacgatgtactgattgaatgggaaaatccatccggatggcttataggattcgattttgatgtatactctgttttaactagtagaggcggtattaccgaggcgaccttgtactttgaaaatgttactgaagaatatataggtaatacatataaatgtcgtggacacaactattattttgaaaaaacccttacaactacagtagtattggag

SEQ ID NO: 17 - protein, 351 aa, Vaccinia virus
MTMKMMVHIYFVSLLLLLFHSYAIDIENEITEFFNKMRDTLPAKDSKWLNPACMFGGTMNDIAALGEPFSAKCPPIEDSLLSHRYKDYVVKWERLEKNRRRQVSNKRVKHGDLWIANYTSKFSNRRYLCTVTTKNGDCVQGIVRSHIRKPPSCIPKTYELGTHDKYGIDLYCGILYAKHYNNITWYKDNKEINIDDIKYSQTGKELIIHNPELEDSGRYDCYVHYDDVRIKNDIVVSRCKILTVIPSQDHRFKLILDPKINVTIGEPANITCTAVSTSLLIDDVLIEWENPSGWLIGFDFDVYSVLTSRGGITEATLYFENVTEEYIGNTYKCRGHNYYFEKTLTTTVVLE

SEQ ID NO: 18 - DNA, 1293 bp, Vaccinia virus
  source 1..1293: mol_type = genomic DNA
gacaattaacgatctttataatatatcgtatccacctaccaaagtatagttgtatttttctcatgcgatgtgtgtaaaaaaactgatattatataaatattttagtgccgtataataaagatgacgatgaaaatgatggtacatatatatttcgtatcattattgttattgctattccacagttacgccatagacatcgaaaatgaaatcacagaattcttcaataaaatgagagatactctaccagctaaagactctaaatggttgaatccagcatgtatgttcggaggcacaatgaatgatatagccgctctaggagagccattcagcgcaaagtgtcctcctattgaagacagtcttttatcgcacagatataaagactatgtggttaaatgggaaaggctagaaaaaaatagacggcgacaggtttctaataaacgtgttaaacatggtgatttatggatagccaactatacatctaaattcagtaaccgtaggtatttgtgcaccgtaactacaaagaatggtgactgtgttcagggtatagttagatctcatattagaaaacctccttcatgcattccaaaaacatatgaactaggtactcatgataagtatggcatagacttatactgtggaattctttacgcaaaacattataataatataacttggtataaagataataaggaaattaatatcgacgacattaagtattcacaaacgggaaaggaattaattattcataatccagagttagaagatagcggaagatacgactgttacgttcattacgacgacgttagaatcaagaatgatatcgtagtatcaagatgtaaaatacttacggttataccgtcacaagaccacaggtttaaactaatactagatccaaaaatcaacgtaacgataggagaacctgccaatataacatgcactgctgtgtcaacgtcattattgattgacgatgtactgattgaatgggaaaatccatccggatggcttataggattcgattttgatgtatactctgttttaactagtagaggcggtattaccgaggcgaccttgtactttgaaaatgttactgaagaatatataggtaatacatataaatgtcgtggacacaactattattttgaaaaaacccttacaactacagtagtattggagtaaatatacaatgcatttttatatacattactgaataattattattattatttatatcgtatttgtgctataacgcgactatctaggtatttgtatctcaccgatagagaacatataaat

SEQ ID NO: 19 - DNA, 33 bp, synthetic construct
  source 1..33: mol_type = other DNA
gcgccatgggccacagttacgccatagacatcg

SEQ ID NO: 20 - DNA, 33 bp, synthetic construct
  source 1..33: mol_type = other DNA
cgcctcgagctccaatactactgtagttgtaag

SEQ ID NO: 21 - DNA, 36 bp, synthetic construct
  source 1..36: mol_type = other DNA
cgcccatgggcccgtcacaagaccacaggtttaaac

SEQ ID NO: 22 - DNA, 33 bp, synthetic construct; identical to SEQ ID NO: 20
  source 1..33: mol_type = other DNA

SEQ ID NO: 23 - DNA, 35 bp, synthetic construct
  source 1..35: mol_type = other DNA
gcgggatcccacaggtttaaactaatactagatcc

SEQ ID NO: 24 - DNA, 35 bp, synthetic construct
  source 1..35: mol_type = other DNA
gcggccgctctccaatactactgtagttgtaaggg

SEQ ID NO: 25 - DNA, 24 bp, synthetic construct
  source 1..24: mol_type = other DNA
gcgccatggcaggatccaaatggg

SEQ ID NO: 26 - DNA, 24 bp, synthetic construct
  source 1..24: mol_type = other DNA
gcggaattcgtcgacggaaccacc

SEQ ID NO: 27 - DNA, 23 bp, synthetic construct
  source 1..23: mol_type = other DNA
cgcggatccgcacagccgccggg

SEQ ID NO: 28 - DNA, 21 bp, synthetic construct
  source 1..21: mol_type = other DNA
cgcgtcgaccctgacatgtcg

SEQ ID NO: 29 - DNA, 25 bp, synthetic construct
  source 1..25: mol_type = other DNA
gcgggatccatagacatcgaaaatg

SEQ ID NO: 30 - DNA, 37 bp, synthetic construct
  source 1..37: mol_type = other DNA
cgcgtcgacttttctaatatgagatctaactataccc

SEQ ID NO: 31 - protein, 100 aa, Ectromelia virus
FKLILDPKINVTIGEPANITCTAVSTSLLVDDVLIDWENPSGWIIGLDFGVYSILTSSGGITEATLYFENVTEEYIGNTYTCRGHNYYFDKTLTTTVVLE

SEQ ID NO: 32 - protein, 100 aa, Monkeypox virus
FKLILDPKINVTIGEPANITCSAVSTSLFVDDVLIEWENPSGWIIGLDFGVYSILTSRGGITEATLYFENVTEEYIGNTYTCRGHNYYFDKTLTTTVVLE

SEQ ID NO: 33 - protein, 100 aa, variola virus
FKLILDSKINVIIGEPANITCTAVSTSLLFDDVLIEWENPSGWLIGFNFDVYSVLTSRGGITEASLYFKNVTEEYIGNTYKCRGHNYYFEKTLTTTVVLE

SEQ ID NO: 34 - protein, 8 aa, synthetic construct
GGGGGGGG

SEQ ID NO: 35 - protein, 46 aa, synthetic construct
AEAAAKEAAAKEAAAKEAAAKALEAEAAAKEAAAKEAAAKEAAAKA

SEQ ID NO: 36 - protein, 20 aa, synthetic construct
APAPAPAPAPAPAPAPAPAP

SEQ ID NO: 37 - DNA, 300 bp, Vaccinia virus
  source 1..300: mol_type = genomic DNA
tttaaactaatactagatccaaaaatcaacgtaacgataggagaacctgccaatataacatgcactgctgtgtcaacgtcattattgattgacgatgtactgattgaatgggaaaatccatccggatggcttataggattcgattttgatgtatactctgttttaactagtagaggcggtattaccgaggcgaccttgtactttgaaaatgttactgaagaatatataggtaatacatataaatgtcgtggacacaactattattttgaaaaaacccttacaactacagtagtattggag